European Patent Application EP 4 382 120 A1, published June 12, 2024. Title: ANTI-SLC1 A4 MONOCLONAL ANTIBODIES AND USES THEREOF. Applicant: INSTITUT REGIONAL DU CANCER DE MONTPELLIER. Application FR. The sequence listing filed with the application follows.

SEQUENCE LISTING (56 sequences)

SEQ ID NO: 1 - protein, 8 aa, synthetic construct
GFTFSNYY

SEQ ID NO: 2 - protein, 8 aa, synthetic construct
YIYGSSRD

SEQ ID NO: 3 - protein, 11 aa, synthetic construct
VRSSNSGGMDV

SEQ ID NO: 4 - protein, 116 aa, synthetic construct
MAEVQLVESGGSLVKPGGSLRLSCAASGFTFSNYYMNWVRQAPGKGLEWISYIYGSSRDIGYADFVKGRFTISRDNAKNSLYLQMNSLRAEDTAVYYCVRSSNSGGMDVWGRGTLV

SEQ ID NO: 5 - protein, 9 aa, synthetic construct
SSDVGGGSD

SEQ ID NO: 6 - skipped

SEQ ID NO: 7 - protein, 10 aa, synthetic construct
SSYTYYSTRV

SEQ ID NO: 8 - protein, 126 aa, synthetic construct
TVSSGGGGSGGGGSGGGGSQSVLTQPASVSGSPGQSITISCAGTSSDVGGGSDVSWYQQHPGKAPKLMIYGDSYRPSGVSNRFSGSKSGNTASLTISGLQAEDEADYYCSSYTYYSTRVFGGGTKL

SEQ ID NO: 9 - protein, 8 aa, synthetic construct
GFTFSNYY

SEQ ID NO: 10 - protein, 8 aa, synthetic construct
SIYGSSRG

SEQ ID NO: 11 - protein, 9 aa, synthetic construct
VRSNYGMDV

SEQ ID NO: 12 - protein, 116 aa, synthetic construct
MAEVQLVESGGSLVKPGGSLRLSCAASGFTFSNYYMNWVRQAPGKGLEWISSIYGSSRGIGYADFVKGRFTISRDNAKNSLYLQMNSLRAEDTAVYYCVRSNYGMDVWGRGTLVTV

SEQ ID NO: 13 - protein, 9 aa, synthetic construct
SSDVGGYSD

SEQ ID NO: 14 - skipped

SEQ ID NO: 15 - protein, 9 aa, synthetic construct
SSSTDYSTR

SEQ ID NO: 16 - protein, 124 aa, synthetic construct
SSGGGGSGGGGSGGGGSQSVLTQPASVSGSPGQSITISCAGTSSDVGGYSDVSWYQQHPGKAPKLMIYSDSQRPSGVSNRFSGSKSGNTASLTISGLQAEDEADYYCSSSTDYSTRVFGGGTKL

SEQ ID NO: 17 - protein, 8 aa, synthetic construct
GFTFSNAY

SEQ ID NO: 18 - protein, 8 aa, synthetic construct
GIYGSSRS

SEQ ID NO: 19 - protein, 12 aa, synthetic construct
VRSSSSYGSGMD

SEQ ID NO: 20 - protein, 117 aa, synthetic construct
MAEVQLVESGGSLVKPGGSLRLSCAASGFTFSNAYMNWVRQAPGKGLEWISGIYGSSRSIYYADFVKGRFTISRDNAKNSLYLQMNSLRAEDTAVYYCVRSSSSYGSGMDVWGRGTL

SEQ ID NO: 21 - protein, 9 aa, synthetic construct
SSDVGGSDD

SEQ ID NO: 22 - skipped

SEQ ID NO: 23 - protein, 10 aa, synthetic construct
SSNTYDSTRV

SEQ ID NO: 24 - protein, 127 aa, synthetic construct
VTVSSGGGGSGGGGSGGGGSQSVLTQPASVSGSPGQSITISCAGTSSDVGGSDDVSWYQQHPGKAPKLMIYGDSNRPSGVSNRFSGSKSGNTASLTISGLQAEDEADYYCSSNTYDSTRVFGGGTKL

SEQ ID NO: 25 - protein, 8 aa, synthetic construct
GFTFSNAA

SEQ ID NO: 26 - protein, 8 aa, synthetic construct
NIQGSSSS

SEQ ID NO: 27 - protein, 13 aa, synthetic construct
VRSSSSYGSGMDV

SEQ ID NO: 28 - protein, 116 aa, synthetic construct
MAEVQLVESGGSLVKPGGSLRLSCAASGFTFSNAAMNWVRQAPGKGLEWISNIQGSSSSIYYADFVKGRFTISRDNAKNSLYLQMNSLRAEDTAVYYCVRSSDDSFGSGMDVWGRG

SEQ ID NO: 29 - protein, 9 aa, synthetic construct
SSDVGGYYS

SEQ ID NO: 30 - skipped

SEQ ID NO: 31 - protein, 10 aa, synthetic construct
SSYTSYSTRV

SEQ ID NO: 32 - protein, 129 aa, synthetic construct
TLVTVSSGGGGSGGGGSGGGGSQSVLTQPASVSGSPGQSITISCAGTSSDVGGYYSVSWYQQHPGKAPKLMIYDDSNRPSGVSNRFSGSKSGNTASLTISGLQAEDEADYYCSSYTSYSTRVFGGGTKL

SEQ ID NO: 33 - protein, 8 aa, synthetic construct
GFTFSNYG

SEQ ID NO: 34 - protein, 8 aa, synthetic construct
SISGSSSS

SEQ ID NO: 35 - protein, 9 aa, synthetic construct
VRSYYGMDV

SEQ ID NO: 36 - protein, 117 aa, synthetic construct
MAEVQLVESGGSLVKPGGSLRLSCAASGFTFSNYGMNWVRQAPGKGLEWISSISGSSSSISYADFVKGRFTISRDNAKNSLYLQMNSLRAEDTAVYYCVRSYYGMDVWGRGTLVTVS

SEQ ID NO: 37 - protein, 9 aa, synthetic construct
SSDVGGYGQ

SEQ ID NO: 38 - skipped

SEQ ID NO: 39 - protein, 10 aa, synthetic construct
SSYTQDSTRV

SEQ ID NO: 40 - protein, 123 aa, synthetic construct
SGGGGSGGGGSGGGGSQSVLTQPASVSGSPGQSITISCAGTSSDVGGYGQVSWYQQHPGKAPKLMIYSDSSRPSGVSNRFSGSKSGNTASLTISGLQAEDEADYYCSSYTQDSTRVFGGGTKL

SEQ ID NO: 41 - protein, 8 aa, synthetic construct
GFTFSNNA

SEQ ID NO: 42 - protein, 8 aa, synthetic construct
YISGSSRN

SEQ ID NO: 43 - protein, 14 aa, synthetic construct
VRSSYYGFGSGMDV

SEQ ID NO: 44 - protein, 116 aa, synthetic construct
MAEVQLVESGGSLVKPGGSLRLSCAASGFTFSNNAMNWVRQAPGKGLEWISYISGSSRNIYYADFVKGRFTISRDNAKNSLYLQMNSLRAEDTAVYYCVRSSYYGFGSGMDVWGRG

SEQ ID NO: 45 - protein, 9 aa, synthetic construct
SSDVGGNSY

SEQ ID NO: 46 - skipped

SEQ ID NO: 47 - protein, 10 aa, synthetic construct
SSNTGYSTRV

SEQ ID NO: 48 - protein, 129 aa, synthetic construct
TLVTVSSGGGGSGGGGSGGGGSQSVLTQPASVSGSPGQSITISCAGTSSDVGGNSYVSWYQQHPGKAPKLMIYYDSQRPSGVSNRFSGSKSGNTASLTISGLQAEDEADYYCSSNTGYSTRVFGGGTKL

SEQ ID NO: 49 - protein, 228 aa, synthetic construct
APSTCSKPTCPPPELLGGPSVFIFPPKPKDTLMISRTPEVTCVVVDVSEDDPEVQFTWYINNEQVRTARPPLREQQFNSTIRVVSTLPIAHEDWLRGKEFKCKVHNKALPAPIEKTISKARGQPLEPKVYTMGPPREELSSRSVSLTCMINGFYPSDISVEWEKNGKAEDNYKTTPAVLDSDGSYFLYSKLSVPTSEWQRGDVFTCSVMHEALHNHYTQKSISRSPGK

SEQ ID NO: 50 - protein, 232 aa, synthetic construct
EPKSCDKTHTCPPCPAPELLGGPSVFLFPPKPKDTLMISRTPEVTCVVVDVSHEDPEVKFNWYVDGVEVHNAKTKPREEQYNSTYRVVSVLTVLHQDWLNGKEYKCKVSNKALPAPIEKTISKAKGQPREPQVYTLPPSRDELTKNQVSLTCLVKGFYPSDIAVEWESNGQPENNYKTTPPVLDSDGSFFLYSKLTVDKSRWQQGNVFSCSVMHEALHNHYTQKSLSLSPGK

SEQ ID NO: 51 - protein, 77 aa, synthetic construct
KPGSGAQTLQSSDLGLEDSGPPPVPKETVDSFLDLARNLFPSNLVVAAFRTYATDYKVVTQNSSSGNVTHEKIPIGT

SEQ ID NO: 52 - protein, 77 aa, synthetic construct
KPGAGAQTLQSSSLGLENSGPPPVSKETVDSFLDLLRNLFPSNLVVAAFTTSATDYTVVTHNTSSGNVTKEKIPVVT

SEQ ID NO: 53 - RNA, 21 nt, synthetic construct
  source 1..21: mol_type = other RNA
ccatgttattcatggaggaat

SEQ ID NO: 54 - protein, 58 aa, synthetic construct
CCGGCCATGTTATTCATGGAGGAATCTCGAGATTCCTCCATGAATAACATGGTTTTTG

SEQ ID NO: 55 - RNA, 58 nt, synthetic construct
  source 1..58: mol_type = other RNA
ccggccatgttattcatggaggaatctcgagattcctccatgaataacatggtttttg

SEQ ID NO: 56 - RNA, 58 nt, synthetic construct
  source 1..58: mol_type = other RNA
aattcaaaaaccatgttattcatggaggaatctcgagattcctccatgaataacatgg